European Patent Application EP 4 186 517 A1, published May 31, 2023. Title: PD-L1 fusion protein and uses thereof. Applicant: Genexine, Inc. The sequence listing filed with the application follows.

SEQUENCE LISTING (35 sequences)

SEQ ID NO: 1 - protein, 290 aa, Artificial Sequence
  amino acid sequence of human PD-L1(Accession number : Q9NZQ7)
MRIFAVFIFMTYWHLLNAFTVTVPKDLYVVEYGSNMTIECKFPVEKQLDLAALIVYWEMEDKNIIQFVHGEEDLKVQHSSYRQRARLLKDQLSLGNAALQITDVKLQDAGVYRCMISYGGADYKRITVKVNAPYNKINQRILVVDPVTSEHELTCQAEGYPKAEVIWTSSDHQVLSGKTTTTNSKREEKLFNVTSTLRINTTTNEIFYCTFRRLDPEENHTAELVIPELPLAHPPNERTHLVILGAILLCLGVALTFIFRLRKGRMMDVKKCGIQDTNSKKQSDTHLEET

SEQ ID NO: 2 - protein, 290 aa, Artificial Sequence
  amino acid sequence of mouse PD-L1 (Accession number : Q9EP73)
MRIFAGIIFTACCHLLRAFTITAPKDLYVVEYGSNVTMECRFPVERELDLLALVVYWEKEDEQVIQFVAGEEDLKPQHSNFRGRASLPKDQLLKGNAALQITDVKLQDAGVYCCIISYGGADYKRITLKVNAPYRKINQRISVDPATSEHELICQAEGYPEAEVIWTNSDHQPVSGKRSVTTSRTEGMLLNVTSSLRVNATANDVFYCTFWRSQPGQNHTAELIIPELPATHPPQNRTHWVLLGSILLFLIVVSTVLLFLRKQVRMLDVEKCGVEDTSSKNRNDTQFEET

SEQ ID NO: 3 - protein, 221 aa, Artificial Sequence [sequence omitted]

SEQ ID NO: 4 - protein, 115 aa, Artificial Sequence
  amino acid sequence of human PD-L1 V like domain(19-133)
FTVTVPKDLYVVEYGSNMTIECKFPVEKQLDLAALIVYWEMEDKNIIQFVHGEEDLKVQHSSYRQRARLLKDQLSLGNAALQITDVKLQDAGVYRCMISYGGADYKRITVKVNAP

SEQ ID NO: 5 - protein, 109 aa, Artificial Sequence
  amino acid sequence of human PD-L1 V like domain(19-127)
FTVTVPKDLYVVEYGSNMTIECKFPVEKQLDLAALIVYWEMEDKNIIQFVHGEEDLKVQHSSYRQRARLLKDQLSLGNAALQITDVKLQDAGVYRCMISYGGADYKRIT

SEQ ID NO: 6 - protein, 107 aa, Artificial Sequence
  amino acid sequence of human PD-L1 V like domain (21-127)
VTVPKDLYVVEYGSNMTIECKFPVEKQLDLAALIVYWEMEDKNIIQFVHGEEDLKVQHSSYRQRARLLKDQLSLGNAALQITDVKLQDAGVYRCMISYGGADYKRIT

SEQ ID NO: 7 - protein, 106 aa, Artificial Sequence
  amino acid sequence containng human PD-L1 C like domain (134-239)
YNKINQRILVVDPVTSEHELTCQAEGYPKAEVIWTSSDHQVLSGKTTTTNSKREEKLFNVTSTLRINTTTNEIFYCTFRRLDPEENHTAELVIPELPLAHPPNERT

SEQ ID NO: 8 - protein, 105 aa, Artificial Sequence
  amino acid sequence including human PD-L1 C like domain (134-238)
YNKINQRILVVDPVTSEHELTCQAEGYPKAEVIWTSSDHQVLSGKTTTTNSKREEKLFNVTSTLRINTTTNEIFYCTFRRLDPEENHTAELVIPELPLAHPPNER

SEQ ID NO: 9 - protein, 107 aa, Artificial Sequence
  amino acid sequence of mouse PD-L1 V like domain(21-127)
ITAPKDLYVVEYGSNVTMECRFPVERELDLLALVVYWEKEDEQVIQFVAGEEDLKPQHSNFRGRASLPKDQLLKGNAALQITDVKLQDAGVYCCIISYGGADYKRIT

SEQ ID NO: 10 - protein, 7 aa, Artificial Sequence
  linker between PD-L1 and Fc
GGGSGGS

SEQ ID NO: 11 - protein, 223 aa, Artificial Sequence
  modified Fc region
THTCPPCPSHTQPLGVFLFPPKPKDTLMISRTPEVTCVVVDVSQEDPEVQFNWYVDGVEVHNAKTKPREEQFNSTYRVVSVLTVLHQDWLNGKEYKCKVSNKGLPSSIEKTISKAKGQPREPQVYTLPPSQEEMTKNQVSLTCLVKGFYPSDIAVEWESNGQPENNYKTTPPVLDSDGSFFLYSRLTVDKSRWQEGNVFSCSVMHEALHNHYTQKSLSLSLGK

SEQ ID NO: 12 - protein, 451 aa, Artificial Sequence
  sPD-L1-hyFc
FTVTVPKDLYVVEYGSNMTIECKFPVEKQLDLAALIVYWEMEDKNIIQFVHGEEDLKVQHSSYRQRARLLKDQLSLGNAALQITDVKLQDAGVYRCMISYGGADYKRITVKVNAPYNKINQRILVVDPVTSEHELTCQAEGYPKAEVIWTSSDHQVLSGKTTTTNSKREEKLFNVTSTLRINTTTNEIFYCTFRRLDPEENHTAELVIPELPLAHPPNERTGGGSGGSTHTCPPCPSHTQPLGVFLFPPKPKDTLMISRTPEVTCVVVDVSQEDPEVQFNWYVDGVEVHNAKTKPREEQFNSTYRVVSVLTVLHQDWLNGKEYKCKVSNKGLPSSIEKTISKAKGQPREPQVYTLPPSQEEMTKNQVSLTCLVKGFYPSDIAVEWESNGQPENNYKTTPPVLDSDGSFFLYSRLTVDKSRWQEGNVFSCSVMHEALHNHYTQKSLSLSLGK

SEQ ID NO: 13 - protein, 345 aa, Artificial Sequence
  sPD-L1 variant-hyFc (PD-L1-GS/IgG1/hyFc)
FTVTVPKDLYVVEYGSNMTIECKFPVEKQLDLAALIVYWEMEDKNIIQFVHGEEDLKVQHSSYRQRARLLKDQLSLGNAALQITDVKLQDAGVYRCMISYGGADYKRITVKVNAPGGGSGGSTHTCPPCPSHTQPLGVFLFPPKPKDTLMISRTPEVTCVVVDVSQEDPEVQFNWYVDGVEVHNAKTKPREEQFNSTYRVVSVLTVLHQDWLNGKEYKCKVSNKGLPSSIEKTISKAKGQPREPQVYTLPPSQEEMTKNQVSLTCLVKGFYPSDIAVEWESNGQPENNYKTTPPVLDSDGSFFLYSRLTVDKSRWQEGNVFSCSVMHEALHNHYTQKSLSLSLGK

SEQ ID NO: 14 - protein, 30 aa, Artificial Sequence
  IgD hinge (from hyFc5)
RNTGRGGEEKKKEKEKEEQEERETKTPECP

SEQ ID NO: 15 - protein, 466 aa, Artificial Sequence
  sPD-L1 variant-hyFc (PD-L1-IgD/hyFc)
FTVTVPKDLYVVEYGSNMTIECKFPVEKQLDLAALIVYWEMEDKNIIQFVHGEEDLKVQHSSYRQRARLLKDQLSLGNAALQITDVKLQDAGVYRCMISYGGADYKRITVKVNAPYNKINQRILVVDPVTSEHELTCQAEGYPKAEVIWTSSDHQVLSGKTTTTNSKREEKLFNVTSTLRINTTTNEIFYCTFRRLDPEENHTAELVIPELPLAHPPNERTRNTGRGGEEKKKEKEKEEQEERETKTPECPSHTQPLGVFLFPPKPKDTLMISRTPEVTCVVVDVSQEDPEVQFNWYVDGVEVHNAKTKPREEQFNSTYRVVSVLTVLHQDWLNGKEYKCKVSNKGLPSSIEKTISKAKGQPREPQVYTLPPSQEEMTKNQVSLTCLVKGFYPSDIAVEWESNGQPENNYKTTPPVLDSDGSFFLYSRLTVDKSRWQEGNVFSCSVMHEALHNHYTQKSLSLSLGK

SEQ ID NO: 16 - protein, 8 aa, Artificial Sequence
  IgG1 hinge (from modified Fc region)
THTCPPCP

SEQ ID NO: 17 - protein, 20 aa, Artificial Sequence
  linker between PD-L1 and Fc
AAGSGGGGGSGGGGSGGGGS

SEQ ID NO: 18 - protein, 5 aa, Artificial Sequence
  linker between PD-L1 and Fc
GGSGG

SEQ ID NO: 19 - protein, 9 aa, Artificial Sequence
  linker between PD-L1 and Fc
GGSGGSGGS

SEQ ID NO: 20 - protein, 6 aa, Artificial Sequence
  linker between PD-L1 and Fc
GGGSGG

SEQ ID NO: 21 - protein, 18 aa, Artificial Sequence
  linker between PD-L1 and Fc
KESGSVSSEQLAQFRSLD

SEQ ID NO: 22 - protein, 14 aa, Artificial Sequence
  linker between PD-L1 and Fc
EGKSSGSGSESKST

SEQ ID NO: 23 - protein, 12 aa, Artificial Sequence
  linker between PD-L1 and Fc
GSAGSAAGSGEF

SEQ ID NO: 24 - protein, 12 aa, Artificial Sequence
  linker between PD-L1 and Fc
CRRRRRREAEAC

SEQ ID NO: 25 - protein, 8 aa, Artificial Sequence
  linker between PD-L1 and Fc
GGGGGGGG

SEQ ID NO: 26 - protein, 6 aa, Artificial Sequence
  linker between PD-L1 and Fc
GGGGGG

SEQ ID NO: 27 - protein, 13 aa, Artificial Sequence
  linker between PD-L1 and Fc
AEAAAKEAAAAKA

SEQ ID NO: 28 - protein, 5 aa, Artificial Sequence
  linker between PD-L1 and Fc
PAPAP

SEQ ID NO: 29 - protein, 17 aa, Artificial Sequence
  linker between PD-L1 and Fc
VSQTSKLTRAETVFPDV

SEQ ID NO: 30 - protein, 6 aa, Artificial Sequence
  linker between PD-L1 and Fc
PLGLWA

SEQ ID NO: 31 - protein, 10 aa, Artificial Sequence
  linker between PD-L1 and Fc
TRHRQPRGWE

SEQ ID NO: 32 - protein, 10 aa, Artificial Sequence
  linker between PD-L1 and Fc
AGNRVRRSVG

SEQ ID NO: 33 - protein, 8 aa, Artificial Sequence
  linker between PD-L1 and Fc
RRRRRRRR

SEQ ID NO: 34 - protein, 4 aa, Artificial Sequence
  linker between PD-L1 and Fc
GFLG

SEQ ID NO: 35 - protein, 31 aa, Artificial Sequence
  linker between PD-L1 and Fc
GSSGGSGSSGGSGGGDEADGSRGSQKAGVDE